European Patent Specification EP 3 266 800 B1, published November 29, 2023. Title: Binding agents directed against the CH1 domain of IgG antibodies. Applicant: Bac IP B.V. The sequence listing filed with the application follows.

SEQUENCE LISTING (217 sequences)

SEQ ID NO: 1 - protein, 129 aa, Artificial
  CH1-7 k0-0
QVQLQESGGGLVQAGGSLRLSCAVSGNTLSRYAMGWFRQTPGNEREFVAAIRWNNGATYYADSVEGRFTISRDSGKNTVYLQMNNLQPEDTAVYYCAGRFLGYASSNAYHEALYNYDYWGQGTQVTVSS

SEQ ID NO: 2 - protein, 129 aa, Artificial
  CH1-7 k0-1
QVQLQESGGGLVQAGGSLRLSCAVSGNTLSRYAMGWFRQTPGNEREFVAAIRWNNGATYYAESVEGRFTISRDSGKNTVYLQMNNLQPEDTAVYYCAGRFLGYASSNAYHEALYNYDYWGQGTQVTVSS

SEQ ID NO: 3 - protein, 129 aa, Artificial
  CH1-7 k0-2
QVQLQESGGGLVQAGGSLRLSCAVSGNTLSRYAMGWFRQTPGNEREFVAAIRWNNGATYYADSVEGRFTISRDTGKNTVYLQMNNLQPEDTAVYYCAGRFLGYASSNAYHEALYNYDYWGQGTQVTVSS

SEQ ID NO: 4 - protein, 129 aa, Artificial
  CH1-7 k0-3
QVQLQESGGGLVQAGGSLRLSCAVSGNTLSRYAMGWFRQTPGNEREFVAAIRWNNGATYYAESVEGRFTISRDTGKNTVYLQMNNLQPEDTAVYYCAGRFLGYASSNAYHEALYNYDYWGQGTQVTVSS

SEQ ID NO: 5 - protein, 129 aa, Artificial
  CH1-7 k0-4
QVQLQESGGGLVQAGGSLRLSCAVSGNTLSRYAMGWFRQTPGNEREFVAAIRWNNGATYYADAVEGRFTISRDSGKNTVYLQMNNLQPEDTAVYYCAGRFLGYASSNAYHEALYNYDYWGQGTQVTVSS

SEQ ID NO: 6 - protein, 129 aa, Artificial
  CH1-7 k0-5
QVQLQESGGGLVQAGGSLRLSCAVSGNTLSRYAMGWFRQTPGNEREFVAAIRWNNGATYYADSVEGRFTISRDNGKNTVYLQMNNLQPEDTAVYYCAGRFLGYASSNAYHEALYNYDYWGQGTQVTVSS

SEQ ID NO: 7 - protein, 129 aa, Artificial
  CH1-7 k0-6
QVQLQESGGGLVQAGGSLRLSCAVSGNTLSRYAMGWFRQTPGNEREFVAAIRWNNGATYYADAVEGRFTISRDNGKNTVYLQMNNLQPEDTAVYYCAGRFLGYASSNAYHEALYNYDYWGQGTQVTVSS

SEQ ID NO: 8 - protein, 129 aa, Artificial
  CH1-7 k0-7
QVQLQESGGGLVQAGGSLRLSCAVSGNTLSRYAMGWFRQTPGNEREFVAAIRWNNGATYYADAVEGRFTISRDTGKNTVYLQMNNLQPEDTAVYYCAGRFLGYASSNAYHEALYNYDYWGQGTQVTVSS

SEQ ID NO: 9 - protein, 129 aa, Artificial
  CH1-7 k0-8
QVQLQESGGGLVQAGGSLRLSCAVSGNTLSRYAMGWFRQTPGNEREFVAAIRWNNGATYYAESVEGRFTISRDNGKNTVYLQMNNLQPEDTAVYYCAGRFLGYASSNAYHEALYNYDYWGQGTQVTVSS

SEQ ID NO: 10 - protein, 129 aa, Artificial
  CH1-7 k1-0
QVQLQESGGGLVQAGGSLRLSCAVSGNTLSRYAMGWFRQTPGKEREFVAAIRWNNGATYYADSVEGRFTISRDSGKNTVYLQMNNLQPEDTAVYYCAGRFLGYASSNAYHEALYNYDYWGQGTQVTVSS

SEQ ID NO: 11 - protein, 129 aa, Artificial
  CH1-7 k1-1
QVQLQESGGGLVQAGGSLRLSCAVSGNTLSRYAMGWFRQTPGKEREFVAAIRWNNGATYYAESVEGRFTISRDSGKNTVYLQMNNLQPEDTAVYYCAGRFLGYASSNAYHEALYNYDYWGQGTQVTVSS

SEQ ID NO: 12 - protein, 129 aa, Artificial
  CH1-7 k1-2
QVQLQESGGGLVQAGGSLRLSCAVSGNTLSRYAMGWFRQTPGKEREFVAAIRWNNGATYYADSVEGRFTISRDTGKNTVYLQMNNLQPEDTAVYYCAGRFLGYASSNAYHEALYNYDYWGQGTQVTVSS

SEQ ID NO: 13 - protein, 129 aa, Artificial
  CH1-7 k1-3
QVQLQESGGGLVQAGGSLRLSCAVSGNTLSRYAMGWFRQTPGKEREFVAAIRWNNGATYYAESVEGRFTISRDTGKNTVYLQMNNLQPEDTAVYYCAGRFLGYASSNAYHEALYNYDYWGQGTQVTVSS

SEQ ID NO: 14 - protein, 129 aa, Artificial
  CH1-7 k1-4
QVQLQESGGGLVQAGGSLRLSCAVSGNTLSRYAMGWFRQTPGKEREFVAAIRWNNGATYYADAVEGRFTISRDSGKNTVYLQMNNLQPEDTAVYYCAGRFLGYASSNAYHEALYNYDYWGQGTQVTVSS

SEQ ID NO: 15 - protein, 129 aa, Artificial
  CH1-7 k1-5
QVQLQESGGGLVQAGGSLRLSCAVSGNTLSRYAMGWFRQTPGKEREFVAAIRWNNGATYYADSVEGRFTISRDNGKNTVYLQMNNLQPEDTAVYYCAGRFLGYASSNAYHEALYNYDYWGQGTQVTVSS

SEQ ID NO: 16 - protein, 129 aa, Artificial
  CH1-7 k1-6
QVQLQESGGGLVQAGGSLRLSCAVSGNTLSRYAMGWFRQTPGKEREFVAAIRWNNGATYYADAVEGRFTISRDNGKNTVYLQMNNLQPEDTAVYYCAGRFLGYASSNAYHEALYNYDYWGQGTQVTVSS

SEQ ID NO: 17 - protein, 129 aa, Artificial
  CH1-7 k1-7
QVQLQESGGGLVQAGGSLRLSCAVSGNTLSRYAMGWFRQTPGKEREFVAAIRWNNGATYYADAVEGRFTISRDTGKNTVYLQMNNLQPEDTAVYYCAGRFLGYASSNAYHEALYNYDYWGQGTQVTVSS

SEQ ID NO: 18 - protein, 129 aa, Artificial
  CH1-7 k1-8
QVQLQESGGGLVQAGGSLRLSCAVSGNTLSRYAMGWFRQTPGKEREFVAAIRWNNGATYYAESVEGRFTISRDNGKNTVYLQMNNLQPEDTAVYYCAGRFLGYASSNAYHEALYNYDYWGQGTQVTVSS

SEQ ID NO: 19 - protein, 129 aa, Artificial
  CH1-7 k2-0
QVQLQESGGGLVQAGGSLRLSCAVSGNTLSRYAMGWFRQTPGNEREFVAAIRWNNGATYYADSVKGRFTISRDSGKNTVYLQMNNLQPEDTAVYYCAGRFLGYASSNAYHEALYNYDYWGQGTQVTVSS

SEQ ID NO: 20 - protein, 129 aa, Artificial
  CH1-7 k2-1
QVQLQESGGGLVQAGGSLRLSCAVSGNTLSRYAMGWFRQTPGNEREFVAAIRWNNGATYYAESVKGRFTISRDSGKNTVYLQMNNLQPEDTAVYYCAGRFLGYASSNAYHEALYNYDYWGQGTQVTVSS

SEQ ID NO: 21 - protein, 129 aa, Artificial
  CH1-7 k2-2
QVQLQESGGGLVQAGGSLRLSCAVSGNTLSRYAMGWFRQTPGNEREFVAAIRWNNGATYYADSVKGRFTISRDTGKNTVYLQMNNLQPEDTAVYYCAGRFLGYASSNAYHEALYNYDYWGQGTQVTVSS

SEQ ID NO: 22 - protein, 129 aa, Artificial
  CH1-7 k2-3
QVQLQESGGGLVQAGGSLRLSCAVSGNTLSRYAMGWFRQTPGNEREFVAAIRWNNGATYYAESVKGRFTISRDTGKNTVYLQMNNLQPEDTAVYYCAGRFLGYASSNAYHEALYNYDYWGQGTQVTVSS

SEQ ID NO: 23 - protein, 129 aa, Artificial
  CH1-7 k2-4
QVQLQESGGGLVQAGGSLRLSCAVSGNTLSRYAMGWFRQTPGNEREFVAAIRWNNGATYYADAVKGRFTISRDSGKNTVYLQMNNLQPEDTAVYYCAGRFLGYASSNAYHEALYNYDYWGQGTQVTVSS

SEQ ID NO: 24 - protein, 129 aa, Artificial
  CH1-7 k2-5
QVQLQESGGGLVQAGGSLRLSCAVSGNTLSRYAMGWFRQTPGNEREFVAAIRWNNGATYYADSVKGRFTISRDNGKNTVYLQMNNLQPEDTAVYYCAGRFLGYASSNAYHEALYNYDYWGQGTQVTVSS

SEQ ID NO: 25 - protein, 129 aa, Artificial
  CH1-7 k2-6
QVQLQESGGGLVQAGGSLRLSCAVSGNTLSRYAMGWFRQTPGNEREFVAAIRWNNGATYYADAVKGRFTISRDNGKNTVYLQMNNLQPEDTAVYYCAGRFLGYASSNAYHEALYNYDYWGQGTQVTVSS

SEQ ID NO: 26 - protein, 129 aa, Artificial
  CH1-7 k2-7
QVQLQESGGGLVQAGGSLRLSCAVSGNTLSRYAMGWFRQTPGNEREFVAAIRWNNGATYYADAVKGRFTISRDTGKNTVYLQMNNLQPEDTAVYYCAGRFLGYASSNAYHEALYNYDYWGQGTQVTVSS

SEQ ID NO: 27 - protein, 129 aa, Artificial
  CH1-7 k2-8
QVQLQESGGGLVQAGGSLRLSCAVSGNTLSRYAMGWFRQTPGNEREFVAAIRWNNGATYYAESVKGRFTISRDNGKNTVYLQMNNLQPEDTAVYYCAGRFLGYASSNAYHEALYNYDYWGQGTQVTVSS

SEQ ID NO: 28 - protein, 129 aa, Artificial
  CH1-7 k3-0
QVQLQESGGGLVQAGGSLRLSCAVSGNTLSRYAMGWFRQTPGNEREFVAAIRWNNGATYYADSVEGRFTISRDSGKNTVYLQMNNLKPEDTAVYYCAGRFLGYASSNAYHEALYNYDYWGQGTQVTVSS

SEQ ID NO: 29 - protein, 129 aa, Artificial
  CH1-7 k3-1
QVQLQESGGGLVQAGGSLRLSCAVSGNTLSRYAMGWFRQTPGNEREFVAAIRWNNGATYYAESVEGRFTISRDSGKNTVYLQMNNLKPEDTAVYYCAGRFLGYASSNAYHEALYNYDYWGQGTQVTVSS

SEQ ID NO: 30 - protein, 129 aa, Artificial
  CH1-7 k3-2
QVQLQESGGGLVQAGGSLRLSCAVSGNTLSRYAMGWFRQTPGNEREFVAAIRWNNGATYYADSVEGRFTISRDTGKNTVYLQMNNLKPEDTAVYYCAGRFLGYASSNAYHEALYNYDYWGQGTQVTVSS

SEQ ID NO: 31 - protein, 129 aa, Artificial
  CH1-7 k3-3
QVQLQESGGGLVQAGGSLRLSCAVSGNTLSRYAMGWFRQTPGNEREFVAAIRWNNGATYYAESVEGRFTISRDTGKNTVYLQMNNLKPEDTAVYYCAGRFLGYASSNAYHEALYNYDYWGQGTQVTVSS

SEQ ID NO: 32 - protein, 129 aa, Artificial
  CH1-7 k3-4
QVQLQESGGGLVQAGGSLRLSCAVSGNTLSRYAMGWFRQTPGNEREFVAAIRWNNGATYYADAVEGRFTISRDSGKNTVYLQMNNLKPEDTAVYYCAGRFLGYASSNAYHEALYNYDYWGQGTQVTVSS

SEQ ID NO: 33 - protein, 129 aa, Artificial
  CH1-7 k3-5
QVQLQESGGGLVQAGGSLRLSCAVSGNTLSRYAMGWFRQTPGNEREFVAAIRWNNGATYYADSVEGRFTISRDNGKNTVYLQMNNLKPEDTAVYYCAGRFLGYASSNAYHEALYNYDYWGQGTQVTVSS

SEQ ID NO: 34 - protein, 129 aa, Artificial
  CH1-7 k3-6
QVQLQESGGGLVQAGGSLRLSCAVSGNTLSRYAMGWFRQTPGNEREFVAAIRWNNGATYYADAVEGRFTISRDNGKNTVYLQMNNLKPEDTAVYYCAGRFLGYASSNAYHEALYNYDYWGQGTQVTVSS

SEQ ID NO: 35 - protein, 129 aa, Artificial
  CH1-7 k3-7
QVQLQESGGGLVQAGGSLRLSCAVSGNTLSRYAMGWFRQTPGNEREFVAAIRWNNGATYYADAVEGRFTISRDTGKNTVYLQMNNLKPEDTAVYYCAGRFLGYASSNAYHEALYNYDYWGQGTQVTVSS

SEQ ID NO: 36 - protein, 129 aa, Artificial
  CH1-7 k3-8
QVQLQESGGGLVQAGGSLRLSCAVSGNTLSRYAMGWFRQTPGNEREFVAAIRWNNGATYYAESVEGRFTISRDNGKNTVYLQMNNLKPEDTAVYYCAGRFLGYASSNAYHEALYNYDYWGQGTQVTVSS

SEQ ID NO: 37 - protein, 129 aa, Artificial
  CH1-7 k4-0
QVQLQESGGGLVQAGGSLRLSCAVSGNTLSRYAMGWFRQTPGKEREFVAAIRWNNGATYYADSVKGRFTISRDSGKNTVYLQMNNLQPEDTAVYYCAGRFLGYASSNAYHEALYNYDYWGQGTQVTVSS

SEQ ID NO: 38 - protein, 129 aa, Artificial
  CH1-7 k4-1
QVQLQESGGGLVQAGGSLRLSCAVSGNTLSRYAMGWFRQTPGKEREFVAAIRWNNGATYYAESVKGRFTISRDSGKNTVYLQMNNLQPEDTAVYYCAGRFLGYASSNAYHEALYNYDYWGQGTQVTVSS

SEQ ID NO: 39 - protein, 129 aa, Artificial
  CH1-7 k4-2
QVQLQESGGGLVQAGGSLRLSCAVSGNTLSRYAMGWFRQTPGKEREFVAAIRWNNGATYYADSVKGRFTISRDTGKNTVYLQMNNLQPEDTAVYYCAGRFLGYASSNAYHEALYNYDYWGQGTQVTVSS

SEQ ID NO: 40 - protein, 129 aa, Artificial
  CH1-7 k4-3
QVQLQESGGGLVQAGGSLRLSCAVSGNTLSRYAMGWFRQTPGKEREFVAAIRWNNGATYYAESVKGRFTISRDTGKNTVYLQMNNLQPEDTAVYYCAGRFLGYASSNAYHEALYNYDYWGQGTQVTVSS

SEQ ID NO: 41 - protein, 129 aa, Artificial
  CH1-7 k4-4
QVQLQESGGGLVQAGGSLRLSCAVSGNTLSRYAMGWFRQTPGKEREFVAAIRWNNGATYYADAVKGRFTISRDSGKNTVYLQMNNLQPEDTAVYYCAGRFLGYASSNAYHEALYNYDYWGQGTQVTVSS

SEQ ID NO: 42 - protein, 129 aa, Artificial
  CH1-7 k4-5
QVQLQESGGGLVQAGGSLRLSCAVSGNTLSRYAMGWFRQTPGKEREFVAAIRWNNGATYYADSVKGRFTISRDNGKNTVYLQMNNLQPEDTAVYYCAGRFLGYASSNAYHEALYNYDYWGQGTQVTVSS

SEQ ID NO: 43 - protein, 129 aa, Artificial
  CH1-7 k4-6
QVQLQESGGGLVQAGGSLRLSCAVSGNTLSRYAMGWFRQTPGKEREFVAAIRWNNGATYYADAVKGRFTISRDNGKNTVYLQMNNLQPEDTAVYYCAGRFLGYASSNAYHEALYNYDYWGQGTQVTVSS

SEQ ID NO: 44 - protein, 129 aa, Artificial
  CH1-7 k4-7
QVQLQESGGGLVQAGGSLRLSCAVSGNTLSRYAMGWFRQTPGKEREFVAAIRWNNGATYYADAVKGRFTISRDTGKNTVYLQMNNLQPEDTAVYYCAGRFLGYASSNAYHEALYNYDYWGQGTQVTVSS

SEQ ID NO: 45 - protein, 129 aa, Artificial
  CH1-7 k4-8
QVQLQESGGGLVQAGGSLRLSCAVSGNTLSRYAMGWFRQTPGKEREFVAAIRWNNGATYYAESVKGRFTISRDNGKNTVYLQMNNLQPEDTAVYYCAGRFLGYASSNAYHEALYNYDYWGQGTQVTVSS

SEQ ID NO: 46 - protein, 129 aa, Artificial
  CH1-7 k5-0
QVQLQESGGGLVQAGGSLRLSCAVSGNTLSRYAMGWFRQTPGKEREFVAAIRWNNGATYYADSVEGRFTISRDSGKNTVYLQMNNLKPEDTAVYYCAGRFLGYASSNAYHEALYNYDYWGQGTQVTVSS

SEQ ID NO: 47 - protein, 129 aa, Artificial
  CH1-7 k5-1
QVQLQESGGGLVQAGGSLRLSCAVSGNTLSRYAMGWFRQTPGKEREFVAAIRWNNGATYYAESVEGRFTISRDSGKNTVYLQMNNLKPEDTAVYYCAGRFLGYASSNAYHEALYNYDYWGQGTQVTVSS

SEQ ID NO: 48 - protein, 129 aa, Artificial
  CH1-7 k5-2
QVQLQESGGGLVQAGGSLRLSCAVSGNTLSRYAMGWFRQTPGKEREFVAAIRWNNGATYYADSVEGRFTISRDTGKNTVYLQMNNLKPEDTAVYYCAGRFLGYASSNAYHEALYNYDYWGQGTQVTVSS

SEQ ID NO: 49 - protein, 129 aa, Artificial
  CH1-7 k5-3
QVQLQESGGGLVQAGGSLRLSCAVSGNTLSRYAMGWFRQTPGKEREFVAAIRWNNGATYYAESVEGRFTISRDTGKNTVYLQMNNLKPEDTAVYYCAGRFLGYASSNAYHEALYNYDYWGQGTQVTVSS

SEQ ID NO: 50 - protein, 129 aa, Artificial
  CH1-7 k5-4
QVQLQESGGGLVQAGGSLRLSCAVSGNTLSRYAMGWFRQTPGKEREFVAAIRWNNGATYYADAVEGRFTISRDSGKNTVYLQMNNLKPEDTAVYYCAGRFLGYASSNAYHEALYNYDYWGQGTQVTVSS

SEQ ID NO: 51 - protein, 129 aa, Artificial
  CH1-7 k5-5
QVQLQESGGGLVQAGGSLRLSCAVSGNTLSRYAMGWFRQTPGKEREFVAAIRWNNGATYYADSVEGRFTISRDNGKNTVYLQMNNLKPEDTAVYYCAGRFLGYASSNAYHEALYNYDYWGQGTQVTVSS

SEQ ID NO: 52 - protein, 129 aa, Artificial
  CH1-7 k5-6
QVQLQESGGGLVQAGGSLRLSCAVSGNTLSRYAMGWFRQTPGKEREFVAAIRWNNGATYYADAVEGRFTISRDNGKNTVYLQMNNLKPEDTAVYYCAGRFLGYASSNAYHEALYNYDYWGQGTQVTVSS

SEQ ID NO: 53 - protein, 129 aa, Artificial
  CH1-7 k5-7
QVQLQESGGGLVQAGGSLRLSCAVSGNTLSRYAMGWFRQTPGKEREFVAAIRWNNGATYYADAVEGRFTISRDTGKNTVYLQMNNLKPEDTAVYYCAGRFLGYASSNAYHEALYNYDYWGQGTQVTVSS

SEQ ID NO: 54 - protein, 129 aa, Artificial
  CH1-7 k5-8
QVQLQESGGGLVQAGGSLRLSCAVSGNTLSRYAMGWFRQTPGKEREFVAAIRWNNGATYYAESVEGRFTISRDNGKNTVYLQMNNLKPEDTAVYYCAGRFLGYASSNAYHEALYNYDYWGQGTQVTVSS

SEQ ID NO: 55 - protein, 129 aa, Artificial
  CH1-7 k6-0
QVQLQESGGGLVQAGGSLRLSCAVSGNTLSRYAMGWFRQTPGNEREFVAAIRWNNGATYYADSVKGRFTISRDSGKNTVYLQMNNLKPEDTAVYYCAGRFLGYASSNAYHEALYNYDYWGQGTQVTVSS

SEQ ID NO: 56 - protein, 129 aa, Artificial
  CH1-7 k6-1
QVQLQESGGGLVQAGGSLRLSCAVSGNTLSRYAMGWFRQTPGNEREFVAAIRWNNGATYYAESVKGRFTISRDSGKNTVYLQMNNLKPEDTAVYYCAGRFLGYASSNAYHEALYNYDYWGQGTQVTVSS

SEQ ID NO: 57 - protein, 129 aa, Artificial
  CH1-7 k6-2
QVQLQESGGGLVQAGGSLRLSCAVSGNTLSRYAMGWFRQTPGNEREFVAAIRWNNGATYYADSVKGRFTISRDTGKNTVYLQMNNLKPEDTAVYYCAGRFLGYASSNAYHEALYNYDYWGQGTQVTVSS

SEQ ID NO: 58 - protein, 129 aa, Artificial
  CH1-7 k6-3
QVQLQESGGGLVQAGGSLRLSCAVSGNTLSRYAMGWFRQTPGNEREFVAAIRWNNGATYYAESVKGRFTISRDTGKNTVYLQMNNLKPEDTAVYYCAGRFLGYASSNAYHEALYNYDYWGQGTQVTVSS

SEQ ID NO: 59 - protein, 129 aa, Artificial
  CH1-7 k6-4
QVQLQESGGGLVQAGGSLRLSCAVSGNTLSRYAMGWFRQTPGNEREFVAAIRWNNGATYYADAVKGRFTISRDSGKNTVYLQMNNLKPEDTAVYYCAGRFLGYASSNAYHEALYNYDYWGQGTQVTVSS

SEQ ID NO: 60 - protein, 129 aa, Artificial
  CH1-7 k6-5
QVQLQESGGGLVQAGGSLRLSCAVSGNTLSRYAMGWFRQTPGNEREFVAAIRWNNGATYYADSVKGRFTISRDNGKNTVYLQMNNLKPEDTAVYYCAGRFLGYASSNAYHEALYNYDYWGQGTQVTVSS

SEQ ID NO: 61 - protein, 129 aa, Artificial
  CH1-7 k6-6
QVQLQESGGGLVQAGGSLRLSCAVSGNTLSRYAMGWFRQTPGNEREFVAAIRWNNGATYYADAVKGRFTISRDNGKNTVYLQMNNLKPEDTAVYYCAGRFLGYASSNAYHEALYNYDYWGQGTQVTVSS

SEQ ID NO: 62 - protein, 129 aa, Artificial
  CH1-7 k6-7
QVQLQESGGGLVQAGGSLRLSCAVSGNTLSRYAMGWFRQTPGNEREFVAAIRWNNGATYYADAVKGRFTISRDTGKNTVYLQMNNLKPEDTAVYYCAGRFLGYASSNAYHEALYNYDYWGQGTQVTVSS

SEQ ID NO: 63 - protein, 129 aa, Artificial
  CH1-7 k6-8
QVQLQESGGGLVQAGGSLRLSCAVSGNTLSRYAMGWFRQTPGNEREFVAAIRWNNGATYYAESVKGRFTISRDNGKNTVYLQMNNLKPEDTAVYYCAGRFLGYASSNAYHEALYNYDYWGQGTQVTVSS

SEQ ID NO: 64 - protein, 129 aa, Artificial
  CH1-7 k7-0
QVQLQESGGGLVQAGGSLRLSCAVSGNTLSRYAMGWFRQTPGKEREFVAAIRWNNGATYYADSVKGRFTISRDSGKNTVYLQMNNLKPEDTAVYYCAGRFLGYASSNAYHEALYNYDYWGQGTQVTVSS

SEQ ID NO: 65 - protein, 129 aa, Artificial
  CH1-7 k7-1
QVQLQESGGGLVQAGGSLRLSCAVSGNTLSRYAMGWFRQTPGKEREFVAAIRWNNGATYYAESVKGRFTISRDSGKNTVYLQMNNLKPEDTAVYYCAGRFLGYASSNAYHEALYNYDYWGQGTQVTVSS

SEQ ID NO: 66 - protein, 129 aa, Artificial
  CH1-7 k7-2
QVQLQESGGGLVQAGGSLRLSCAVSGNTLSRYAMGWFRQTPGKEREFVAAIRWNNGATYYADSVKGRFTISRDTGKNTVYLQMNNLKPEDTAVYYCAGRFLGYASSNAYHEALYNYDYWGQGTQVTVSS

SEQ ID NO: 67 - protein, 129 aa, Artificial
  CH1-7 k7-3
QVQLQESGGGLVQAGGSLRLSCAVSGNTLSRYAMGWFRQTPGKEREFVAAIRWNNGATYYAESVKGRFTISRDTGKNTVYLQMNNLKPEDTAVYYCAGRFLGYASSNAYHEALYNYDYWGQGTQVTVSS

SEQ ID NO: 68 - protein, 129 aa, Artificial
  CH1-7 k7-4
QVQLQESGGGLVQAGGSLRLSCAVSGNTLSRYAMGWFRQTPGKEREFVAAIRWNNGATYYADAVKGRFTISRDSGKNTVYLQMNNLKPEDTAVYYCAGRFLGYASSNAYHEALYNYDYWGQGTQVTVSS

SEQ ID NO: 69 - protein, 129 aa, Artificial
  CH1-7 k7-5
QVQLQESGGGLVQAGGSLRLSCAVSGNTLSRYAMGWFRQTPGKEREFVAAIRWNNGATYYADSVKGRFTISRDNGKNTVYLQMNNLKPEDTAVYYCAGRFLGYASSNAYHEALYNYDYWGQGTQVTVSS

SEQ ID NO: 70 - protein, 129 aa, Artificial
  CH1-7 k7-6
QVQLQESGGGLVQAGGSLRLSCAVSGNTLSRYAMGWFRQTPGKEREFVAAIRWNNGATYYADAVKGRFTISRDNGKNTVYLQMNNLKPEDTAVYYCAGRFLGYASSNAYHEALYNYDYWGQGTQVTVSS

SEQ ID NO: 71 - protein, 129 aa, Artificial
  CH1-7 k7-7
QVQLQESGGGLVQAGGSLRLSCAVSGNTLSRYAMGWFRQTPGKEREFVAAIRWNNGATYYADAVKGRFTISRDTGKNTVYLQMNNLKPEDTAVYYCAGRFLGYASSNAYHEALYNYDYWGQGTQVTVSS

SEQ ID NO: 72 - protein, 129 aa, Artificial
  CH1-7 k7-8
QVQLQESGGGLVQAGGSLRLSCAVSGNTLSRYAMGWFRQTPGKEREFVAAIRWNNGATYYAESVKGRFTISRDNGKNTVYLQMNNLKPEDTAVYYCAGRFLGYASSNAYHEALYNYDYWGQGTQVTVSS

SEQ ID NO: 73 - protein, 129 aa, Artificial
  CH1-7 k8-0
QVQLQESGGGLVQAGGSLRLSCAVSGNTLSRYAMGWFRQTPGNEREFVAAIRWNNGATYYADSVKGRFTISRDSGRNTVYLQMNNLKPEDTAVYYCAGRFLGYASSNAYHEALYNYDYWGQGTQVTVSS

SEQ ID NO: 74 - protein, 129 aa, Artificial
  CH1-7 k8-1
QVQLQESGGGLVQAGGSLRLSCAVSGNTLSRYAMGWFRQTPGNEREFVAAIRWNNGATYYAESVKGRFTISRDSGRNTVYLQMNNLKPEDTAVYYCAGRFLGYASSNAYHEALYNYDYWGQGTQVTVSS

SEQ ID NO: 75 - protein, 129 aa, Artificial
  CH1-7 k8-2
QVQLQESGGGLVQAGGSLRLSCAVSGNTLSRYAMGWFRQTPGNEREFVAAIRWNNGATYYADSVKGRFTISRDTGRNTVYLQMNNLKPEDTAVYYCAGRFLGYASSNAYHEALYNYDYWGQGTQVTVSS

SEQ ID NO: 76 - protein, 129 aa, Artificial
  CH1-7 k8-3
QVQLQESGGGLVQAGGSLRLSCAVSGNTLSRYAMGWFRQTPGNEREFVAAIRWNNGATYYAESVKGRFTISRDTGRNTVYLQMNNLKPEDTAVYYCAGRFLGYASSNAYHEALYNYDYWGQGTQVTVSS

SEQ ID NO: 77 - protein, 129 aa, Artificial
  CH1-7 k8-4
QVQLQESGGGLVQAGGSLRLSCAVSGNTLSRYAMGWFRQTPGNEREFVAAIRWNNGATYYADAVKGRFTISRDSGRNTVYLQMNNLKPEDTAVYYCAGRFLGYASSNAYHEALYNYDYWGQGTQVTVSS

SEQ ID NO: 78 - protein, 129 aa, Artificial
  CH1-7 k8-5
QVQLQESGGGLVQAGGSLRLSCAVSGNTLSRYAMGWFRQTPGNEREFVAAIRWNNGATYYADSVKGRFTISRDNGRNTVYLQMNNLKPEDTAVYYCAGRFLGYASSNAYHEALYNYDYWGQGTQVTVSS

SEQ ID NO: 79 - protein, 129 aa, Artificial
  CH1-7 k8-6
QVQLQESGGGLVQAGGSLRLSCAVSGNTLSRYAMGWFRQTPGNEREFVAAIRWNNGATYYADAVKGRFTISRDNGRNTVYLQMNNLKPEDTAVYYCAGRFLGYASSNAYHEALYNYDYWGQGTQVTVSS

SEQ ID NO: 80 - protein, 129 aa, Artificial
  CH1-7 k8-7
QVQLQESGGGLVQAGGSLRLSCAVSGNTLSRYAMGWFRQTPGNEREFVAAIRWNNGATYYADAVKGRFTISRDTGRNTVYLQMNNLKPEDTAVYYCAGRFLGYASSNAYHEALYNYDYWGQGTQVTVSS

SEQ ID NO: 81 - protein, 129 aa, Artificial
  CH1-7 k8-8
QVQLQESGGGLVQAGGSLRLSCAVSGNTLSRYAMGWFRQTPGNEREFVAAIRWNNGATYYAESVKGRFTISRDNGRNTVYLQMNNLKPEDTAVYYCAGRFLGYASSNAYHEALYNYDYWGQGTQVTVSS

SEQ ID NO: 82 - protein, 129 aa, Artificial
  CH1-1
QVQLQESGGGLVQAGGSLRLSCAVSGNTLSRYAMGWFRQAPGNEREFVAAIRWNNGNTYYADSVKGRFTISRDSAKNTVFLQMNSLQPEDTAVYFCAARFLPYASSNAYHEALYNYDYWGQGTQVTVSS

SEQ ID NO: 83 - protein, 129 aa, Artificial
  CH1-2
QVQLQDSGGGLVQAGGSLRLSCAVSGNTLSRYAMGWFRQAPGNEREFVAAIRWNNGNTYYADSVEGRFTISRDSAKNTVYLQMNSLQPEDTAVYYCAARFLPYASSNAYHEALYNYDYWGQGTQVTVSS

SEQ ID NO: 84 - protein, 129 aa, Artificial
  CH1-3
QVQLQDSGGGLVQAGGSLRLSCAVSGNTLSRYAMGWFRQAPGNEREFVAAIRWNNGNTYYADSVKGRFTISRDSAKNTVYLQMNSLQPEDTAVYYCAARFLPYASSNAYHEALYNYDYWGQGTQVTVSS

SEQ ID NO: 85 - protein, 129 aa, Artificial
  CH1-4
QVQLQESGGGLVQAGGSLRLSCAVSGNTLSRYAMGWFRQAPGNEREFVAAIRWNNGATYYADSVEGRFTISRDSGKNTVYLQMNSLQPEDTAVYYCAGRFLGYASSNAYHEALYNYDYWGQGTQVTVSS

SEQ ID NO: 86 - protein, 129 aa, Artificial
  CH1-5
QVQLQDSGGGSVQAGGSLRLSCAVSGNTLSRYAMGWFRQAPGNEREFVAAIRWNNGNTYYADSVKGRFTISRDSAKNTVYLQMNSLQPEDTAVYFCAARFLPYASSNAYHEALYNYDYWGQGTQVTVSS

SEQ ID NO: 87 - protein, 129 aa, Artificial
  CH1-6
QVQLQESGGGLVQAGASLRLSCEVSGNTLSQYAMGWFRQVPGHKREFVAAIRWTNGNTYYADSVEGRFTISRDSAKKTVYLQMNSLQPDDTAIYYCAARFLPYASSNAYHESLYNYDYWGQGTQVTVSS

SEQ ID NO: 88 - protein, 129 aa, Artificial
  CH1-8
QVQLQESGGGSVQAGGSLRLSCAVSGNTLSRYAMGWFRQAPGNEREFVAAIRWNNGNTYYADSVEGRFTISRYSAKNLVYLQMNSLQAEDTAIYYCAARFLPYASSNAYHEALYNYDYWGQGTQVTVSS

SEQ ID NO: 89 - protein, 129 aa, Artificial
  CH1-9
QVQLQESGGGLVQAGGSLRLSCAVSGNTLSRYAMGWFRQAPGNEREFVAAIRWNNGNTYYADSVKGRFTISRDSAKNTVYLQMNSLQPEDTAVYYCASRFLPYASSNAYHEALYNYDYWGQGTQVTVSS

SEQ ID NO: 90 - protein, 129 aa, Artificial
  13_A12
QVQLQDSGGGLVQAGGSLRLSCAVSGNTLSRYATGWFRQAPGNEREFVAAIRWNNGNTYYADSVEGRFTIARDSARDTVYLQMNNLQPEDTAVYYCAARFLPYASSNAYHEALYNYDYWGQGTQVTVSS

SEQ ID NO: 91 - protein, 129 aa, Artificial
  12_A9
QVQLQESGGGSVQAEGSLRLSCAVSGNTLSRYAMGWFRQAPGNEREFVAAIRWNSGHTYYADSVEGRFTISRDSAKNTVYLQMDMLQPEDTAVYYCAARFLPYASSNAYHEALYNYDYWGQGTQVTVSS

SEQ ID NO: 92 - protein, 129 aa, Artificial
  07_E8
QVQLQDSGGGLVQAGGSLTLSCVVSGNTLSRYAMGWFRQAPGNEREFVAAIRWENGNTYYADSVEGRFTISRDSAKNTVYLQMNSLQPEDTAVYYCAARFLPYASSNAYHETLYNYDYWGQGTQVTVSS

SEQ ID NO: 93 - protein, 129 aa, Artificial
  10_F1
QVQLQESGGGLVQAGGSLRLSCAVSGNTLSQYAMGWFRQAPGNEREFVAAIRWNNGNTYYADSVEGRFTISRDSAKNTVYLQMNSLQPEDTAVYYCAARFLPYASSNAYHETLYNYDYWGQGTQVTVSS

SEQ ID NO: 94 - protein, 129 aa, Artificial
  10_F9
QVQLQESGGGLVQAGGSLRLSCAVSGNTLSRYAMGWFRQVLGNEREFVAAIRWNNGNTYYADSVEGRFTISRDSAKNTVYLQMNSLQPEDTAVYYCAARFLPYASSNAYHESLYNYDYWGQGTQVTVSS

SEQ ID NO: 95 - protein, 129 aa, Artificial
  07_F7
QVQLQESGGGLVQAGGSLRLSCAVSGNTLSPYAMGWFRQTPRNEREFVAPIRWNNGNTYYADSVEGRFTISRDSAKNTVYLQMNSLQPEDTAVYYCAARFLPYASSNAYHEALYNYDYWGQGTQVTVSS

SEQ ID NO: 96 - protein, 129 aa, Artificial
  CH1-7k1-9
QVQLQESGGGLVQAGGSLRLSCAVSGNTLSRYAMGWFRQTPGKEREFVAAIRWNNGATYYADSVEGRFTISRDNAKNTVYLQMNNLQPEDTAVYYCAGRFLGYASSNAYHEALYNYDYWGQGTQVTVSS

SEQ ID NO: 97 - protein, 129 aa, Artificial
  CH1-7k1-10
QVQLQESGGGLVQAGGSLRLSCAVSGNTLSRYAMGWFRQTPGKEREFVAAIRWNNGATYYADAVEGRFTISRDNAKNTVYLQMNNLQPEDTAVYYCAGRFLGYASSNAYHEALYNYDYWGQGTQVTVSS

SEQ ID NO: 98 - protein, 129 aa, Artificial
  CH1-7k1-11
QVQLQESGGGLVQAGGSLRLSCAVSGNTLSRYAMGWFRQTPGKEREFVAAIRWNNGATYYAESVEGRFTISRDNAKNTVYLQMNNLQPEDTAVYYCAGRFLGYASSNAYHEALYNYDYWGQGTQVTVSS

SEQ ID NO: 99 - protein, 129 aa, Artificial
  CH1-7k1-12
QVQLQESGGGLVQAGGSLRLSCAVSGNTLSRYAMGWFRQTPGKEREFVAAIRWNNAATYYADSVEGRFTISRDSGKNTVYLQMNNLQPEDTAVYYCAGRFLGYASSNAYHEALYNYDYWGQGTQVTVSS

SEQ ID NO: 100 - protein, 129 aa, Artificial
  CH1-7k1-13
QVQLQESGGGLVQAGGSLRLSCAVSGNTLSRYAMGWFRQTPGKEREFVAAIRWNNAATYYAESVEGRFTISRDSGKNTVYLQMNNLQPEDTAVYYCAGRFLGYASSNAYHEALYNYDYWGQGTQVTVSS

SEQ ID NO: 101 - protein, 129 aa, Artificial
  CH1-7k1-14
QVQLQESGGGLVQAGGSLRLSCAVSGNTLSRYAMGWFRQTPGKEREFVAAIRWNNAATYYADSVEGRFTISRDTGKNTVYLQMNNLQPEDTAVYYCAGRFLGYASSNAYHEALYNYDYWGQGTQVTVSS

SEQ ID NO: 102 - protein, 129 aa, Artificial
  CH1-7k1-15
QVQLQESGGGLVQAGGSLRLSCAVSGNTLSRYAMGWFRQTPGKEREFVAAIRWNNAATYYAESVEGRFTISRDTGKNTVYLQMNNLQPEDTAVYYCAGRFLGYASSNAYHEALYNYDYWGQGTQVTVSS

SEQ ID NO: 103 - protein, 129 aa, Artificial
  CH1-7k1-16
QVQLQESGGGLVQAGGSLRLSCAVSGNTLSRYAMGWFRQTPGKEREFVAAIRWNNAATYYADAVEGRFTISRDSGKNTVYLQMNNLQPEDTAVYYCAGRFLGYASSNAYHEALYNYDYWGQGTQVTVSS

SEQ ID NO: 104 - protein, 129 aa, Artificial
  CH1-7k1-17
QVQLQESGGGLVQAGGSLRLSCAVSGNTLSRYAMGWFRQTPGKEREFVAAIRWNNAATYYADSVEGRFTISRDNAKNTVYLQMNNLQPEDTAVYYCAGRFLGYASSNAYHEALYNYDYWGQGTQVTVSS

SEQ ID NO: 105 - protein, 129 aa, Artificial
  CH1-7k1-18
QVQLQESGGGLVQAGGSLRLSCAVSGNTLSRYAMGWFRQTPGKEREFVAAIRWNNAATYYADAVEGRFTISRDNAKNTVYLQMNNLQPEDTAVYYCAGRFLGYASSNAYHEALYNYDYWGQGTQVTVSS

SEQ ID NO: 106 - protein, 129 aa, Artificial
  CH1-7k1-19
QVQLQESGGGLVQAGGSLRLSCAVSGNTLSRYAMGWFRQTPGKEREFVAAIRWNNAATYYADAVEGRFTISRDTGKNTVYLQMNNLQPEDTAVYYCAGRFLGYASSNAYHEALYNYDYWGQGTQVTVSS

SEQ ID NO: 107 - protein, 129 aa, Artificial
  CH1-7k1-20
QVQLQESGGGLVQAGGSLRLSCAVSGNTLSRYAMGWFRQTPGKEREFVAAIRWNNAATYYAESVEGRFTISRDNAKNTVYLQMNNLQPEDTAVYYCAGRFLGYASSNAYHEALYNYDYWGQGTQVTVSS

SEQ ID NO: 108 - protein, 129 aa, Artificial
  CH1-7k1-21
QVQLQESGGGLVQAGGSLRLSCAVSGNTLSRYAMGWFRQTPGKEREFVAAIRWNEGATYYADSVEGRFTISRDSGKNTVYLQMNNLQPEDTAVYYCAGRFLGYASSNAYHEALYNYDYWGQGTQVTVSS

SEQ ID NO: 109 - protein, 129 aa, Artificial
  CH1-7k1-22
QVQLQESGGGLVQAGGSLRLSCAVSGNTLSRYAMGWFRQTPGKEREFVAAIRWNEGATYYAESVEGRFTISRDSGKNTVYLQMNNLQPEDTAVYYCAGRFLGYASSNAYHEALYNYDYWGQGTQVTVSS

SEQ ID NO: 110 - protein, 129 aa, Artificial
  CH1-7k1-23
QVQLQESGGGLVQAGGSLRLSCAVSGNTLSRYAMGWFRQTPGKEREFVAAIRWNEGATYYADSVEGRFTISRDTGKNTVYLQMNNLQPEDTAVYYCAGRFLGYASSNAYHEALYNYDYWGQGTQVTVSS

SEQ ID NO: 111 - protein, 129 aa, Artificial
  CH1-7k1-24
QVQLQESGGGLVQAGGSLRLSCAVSGNTLSRYAMGWFRQTPGKEREFVAAIRWNEGATYYAESVEGRFTISRDTGKNTVYLQMNNLQPEDTAVYYCAGRFLGYASSNAYHEALYNYDYWGQGTQVTVSS

SEQ ID NO: 112 - protein, 129 aa, Artificial
  CH1-7k1-25
QVQLQESGGGLVQAGGSLRLSCAVSGNTLSRYAMGWFRQTPGKEREFVAAIRWNEGATYYADAVEGRFTISRDSGKNTVYLQMNNLQPEDTAVYYCAGRFLGYASSNAYHEALYNYDYWGQGTQVTVSS

SEQ ID NO: 113 - protein, 129 aa, Artificial
  CH1-7k1-26
QVQLQESGGGLVQAGGSLRLSCAVSGNTLSRYAMGWFRQTPGKEREFVAAIRWNEGATYYADSVEGRFTISRDNAKNTVYLQMNNLQPEDTAVYYCAGRFLGYASSNAYHEALYNYDYWGQGTQVTVSS

SEQ ID NO: 114 - protein, 129 aa, Artificial
  CH1-7k1-27
QVQLQESGGGLVQAGGSLRLSCAVSGNTLSRYAMGWFRQTPGKEREFVAAIRWNEGATYYADAVEGRFTISRDNAKNTVYLQMNNLQPEDTAVYYCAGRFLGYASSNAYHEALYNYDYWGQGTQVTVSS

SEQ ID NO: 115 - protein, 129 aa, Artificial
  CH1-7k1-28
QVQLQESGGGLVQAGGSLRLSCAVSGNTLSRYAMGWFRQTPGKEREFVAAIRWNEGATYYADAVEGRFTISRDTGKNTVYLQMNNLQPEDTAVYYCAGRFLGYASSNAYHEALYNYDYWGQGTQVTVSS

SEQ ID NO: 116 - protein, 129 aa, Artificial
  CH1-7k1-29
QVQLQESGGGLVQAGGSLRLSCAVSGNTLSRYAMGWFRQTPGKEREFVAAIRWNEGATYYAESVEGRFTISRDNAKNTVYLQMNNLQPEDTAVYYCAGRFLGYASSNAYHEALYNYDYWGQGTQVTVSS

SEQ ID NO: 117 - protein, 129 aa, Artificial
  CH1-7k3-9
QVQLQESGGGLVQAGGSLRLSCAVSGNTLSRYAMGWFRQTPGNEREFVAAIRWNNGATYYADSVEGRFTISRDNAKNTVYLQMNNLKPEDTAVYYCAGRFLGYASSNAYHEALYNYDYWGQGTQVTVSS

SEQ ID NO: 118 - protein, 129 aa, Artificial
  CH1-7k3-10
QVQLQESGGGLVQAGGSLRLSCAVSGNTLSRYAMGWFRQTPGNEREFVAAIRWNNGATYYADAVEGRFTISRDNAKNTVYLQMNNLKPEDTAVYYCAGRFLGYASSNAYHEALYNYDYWGQGTQVTVSS

SEQ ID NO: 119 - protein, 129 aa, Artificial
  CH1-7k3-11
QVQLQESGGGLVQAGGSLRLSCAVSGNTLSRYAMGWFRQTPGNEREFVAAIRWNNGATYYAESVEGRFTISRDNAKNTVYLQMNNLKPEDTAVYYCAGRFLGYASSNAYHEALYNYDYWGQGTQVTVSS

SEQ ID NO: 120 - protein, 129 aa, Artificial
  CH1-7k3-12
QVQLQESGGGLVQAGGSLRLSCAVSGNTLSRYAMGWFRQTPGNEREFVAAIRWNNAATYYADSVEGRFTISRDSGKNTVYLQMNNLKPEDTAVYYCAGRFLGYASSNAYHEALYNYDYWGQGTQVTVSS

SEQ ID NO: 121 - protein, 129 aa, Artificial
  CH1-7k3-13
QVQLQESGGGLVQAGGSLRLSCAVSGNTLSRYAMGWFRQTPGNEREFVAAIRWNNAATYYAESVEGRFTISRDSGKNTVYLQMNNLKPEDTAVYYCAGRFLGYASSNAYHEALYNYDYWGQGTQVTVSS

SEQ ID NO: 122 - protein, 129 aa, Artificial
  CH1-7k3-14
QVQLQESGGGLVQAGGSLRLSCAVSGNTLSRYAMGWFRQTPGNEREFVAAIRWNNAATYYADSVEGRFTISRDTGKNTVYLQMNNLKPEDTAVYYCAGRFLGYASSNAYHEALYNYDYWGQGTQVTVSS

SEQ ID NO: 123 - protein, 129 aa, Artificial
  CH1-7k3-15
QVQLQESGGGLVQAGGSLRLSCAVSGNTLSRYAMGWFRQTPGNEREFVAAIRWNNAATYYAESVEGRFTISRDTGKNTVYLQMNNLKPEDTAVYYCAGRFLGYASSNAYHEALYNYDYWGQGTQVTVSS

SEQ ID NO: 124 - protein, 129 aa, Artificial
  CH1-7k3-16
QVQLQESGGGLVQAGGSLRLSCAVSGNTLSRYAMGWFRQTPGNEREFVAAIRWNNAATYYADAVEGRFTISRDSGKNTVYLQMNNLKPEDTAVYYCAGRFLGYASSNAYHEALYNYDYWGQGTQVTVSS

SEQ ID NO: 125 - protein, 129 aa, Artificial
  CH1-7k3-17
QVQLQESGGGLVQAGGSLRLSCAVSGNTLSRYAMGWFRQTPGNEREFVAAIRWNNAATYYADSVEGRFTISRDNAKNTVYLQMNNLKPEDTAVYYCAGRFLGYASSNAYHEALYNYDYWGQGTQVTVSS

SEQ ID NO: 126 - protein, 129 aa, Artificial
  CH1-7k3-18
QVQLQESGGGLVQAGGSLRLSCAVSGNTLSRYAMGWFRQTPGNEREFVAAIRWNNAATYYADAVEGRFTISRDNAKNTVYLQMNNLKPEDTAVYYCAGRFLGYASSNAYHEALYNYDYWGQGTQVTVSS

SEQ ID NO: 127 - protein, 129 aa, Artificial
  CH1-7k3-19
QVQLQESGGGLVQAGGSLRLSCAVSGNTLSRYAMGWFRQTPGNEREFVAAIRWNNAATYYADAVEGRFTISRDTGKNTVYLQMNNLKPEDTAVYYCAGRFLGYASSNAYHEALYNYDYWGQGTQVTVSS

SEQ ID NO: 128 - protein, 129 aa, Artificial
  CH1-7k3-20
QVQLQESGGGLVQAGGSLRLSCAVSGNTLSRYAMGWFRQTPGNEREFVAAIRWNNAATYYAESVEGRFTISRDNAKNTVYLQMNNLKPEDTAVYYCAGRFLGYASSNAYHEALYNYDYWGQGTQVTVSS

SEQ ID NO: 129 - protein, 129 aa, Artificial
  CH1-7k3-21
QVQLQESGGGLVQAGGSLRLSCAVSGNTLSRYAMGWFRQTPGNEREFVAAIRWNEGATYYADSVEGRFTISRDSGKNTVYLQMNNLKPEDTAVYYCAGRFLGYASSNAYHEALYNYDYWGQGTQVTVSS

SEQ ID NO: 130 - protein, 129 aa, Artificial
  CH1-7k3-22
QVQLQESGGGLVQAGGSLRLSCAVSGNTLSRYAMGWFRQTPGNEREFVAAIRWNEGATYYAESVEGRFTISRDSGKNTVYLQMNNLKPEDTAVYYCAGRFLGYASSNAYHEALYNYDYWGQGTQVTVSS

SEQ ID NO: 131 - protein, 129 aa, Artificial
  CH1-7k3-23
QVQLQESGGGLVQAGGSLRLSCAVSGNTLSRYAMGWFRQTPGNEREFVAAIRWNEGATYYADSVEGRFTISRDTGKNTVYLQMNNLKPEDTAVYYCAGRFLGYASSNAYHEALYNYDYWGQGTQVTVSS

SEQ ID NO: 132 - protein, 129 aa, Artificial
  CH1-7k3-24
QVQLQESGGGLVQAGGSLRLSCAVSGNTLSRYAMGWFRQTPGNEREFVAAIRWNEGATYYAESVEGRFTISRDTGKNTVYLQMNNLKPEDTAVYYCAGRFLGYASSNAYHEALYNYDYWGQGTQVTVSS

SEQ ID NO: 133 - protein, 129 aa, Artificial
  CH1-7k3-25
QVQLQESGGGLVQAGGSLRLSCAVSGNTLSRYAMGWFRQTPGNEREFVAAIRWNEGATYYADAVEGRFTISRDSGKNTVYLQMNNLKPEDTAVYYCAGRFLGYASSNAYHEALYNYDYWGQGTQVTVSS

SEQ ID NO: 134 - protein, 129 aa, Artificial
  CH1-7k3-26
QVQLQESGGGLVQAGGSLRLSCAVSGNTLSRYAMGWFRQTPGNEREFVAAIRWNEGATYYADSVEGRFTISRDNAKNTVYLQMNNLKPEDTAVYYCAGRFLGYASSNAYHEALYNYDYWGQGTQVTVSS

SEQ ID NO: 135 - protein, 129 aa, Artificial
  CH1-7k3-27
QVQLQESGGGLVQAGGSLRLSCAVSGNTLSRYAMGWFRQTPGNEREFVAAIRWNEGATYYADAVEGRFTISRDNAKNTVYLQMNNLKPEDTAVYYCAGRFLGYASSNAYHEALYNYDYWGQGTQVTVSS

SEQ ID NO: 136 - protein, 129 aa, Artificial
  CH1-7k3-28
QVQLQESGGGLVQAGGSLRLSCAVSGNTLSRYAMGWFRQTPGNEREFVAAIRWNEGATYYADAVEGRFTISRDTGKNTVYLQMNNLKPEDTAVYYCAGRFLGYASSNAYHEALYNYDYWGQGTQVTVSS

SEQ ID NO: 137 - protein, 129 aa, Artificial
  CH1-7k3-29
QVQLQESGGGLVQAGGSLRLSCAVSGNTLSRYAMGWFRQTPGNEREFVAAIRWNEGATYYAESVEGRFTISRDNAKNTVYLQMNNLKPEDTAVYYCAGRFLGYASSNAYHEALYNYDYWGQGTQVTVSS

SEQ ID NO: 138 - protein, 129 aa, Artificial
  CH1-7k5-9
QVQLQESGGGLVQAGGSLRLSCAVSGNTLSRYAMGWFRQTPGKEREFVAAIRWNNGATYYADSVEGRFTISRDNAKNTVYLQMNNLKPEDTAVYYCAGRFLGYASSNAYHEALYNYDYWGQGTQVTVSS

SEQ ID NO: 139 - protein, 129 aa, Artificial
  CH1-7k5-10
QVQLQESGGGLVQAGGSLRLSCAVSGNTLSRYAMGWFRQTPGKEREFVAAIRWNNGATYYADAVEGRFTISRDNAKNTVYLQMNNLKPEDTAVYYCAGRFLGYASSNAYHEALYNYDYWGQGTQVTVSS

SEQ ID NO: 140 - protein, 129 aa, Artificial
  CH1-7k5-11
QVQLQESGGGLVQAGGSLRLSCAVSGNTLSRYAMGWFRQTPGKEREFVAAIRWNNGATYYAESVEGRFTISRDNAKNTVYLQMNNLKPEDTAVYYCAGRFLGYASSNAYHEALYNYDYWGQGTQVTVSS

SEQ ID NO: 141 - protein, 129 aa, Artificial
  CH1-7k5-12
QVQLQESGGGLVQAGGSLRLSCAVSGNTLSRYAMGWFRQTPGKEREFVAAIRWNNAATYYADSVEGRFTISRDSGKNTVYLQMNNLKPEDTAVYYCAGRFLGYASSNAYHEALYNYDYWGQGTQVTVSS

SEQ ID NO: 142 - protein, 129 aa, Artificial
  CH1-7k5-13
QVQLQESGGGLVQAGGSLRLSCAVSGNTLSRYAMGWFRQTPGKEREFVAAIRWNNAATYYAESVEGRFTISRDSGKNTVYLQMNNLKPEDTAVYYCAGRFLGYASSNAYHEALYNYDYWGQGTQVTVSS

SEQ ID NO: 143 - protein, 129 aa, Artificial
  CH1-7k5-14
QVQLQESGGGLVQAGGSLRLSCAVSGNTLSRYAMGWFRQTPGKEREFVAAIRWNNAATYYADSVEGRFTISRDTGKNTVYLQMNNLKPEDTAVYYCAGRFLGYASSNAYHEALYNYDYWGQGTQVTVSS

SEQ ID NO: 144 - protein, 129 aa, Artificial
  CH1-7k5-15
QVQLQESGGGLVQAGGSLRLSCAVSGNTLSRYAMGWFRQTPGKEREFVAAIRWNNAATYYAESVEGRFTISRDTGKNTVYLQMNNLKPEDTAVYYCAGRFLGYASSNAYHEALYNYDYWGQGTQVTVSS

SEQ ID NO: 145 - protein, 129 aa, Artificial
  CH1-7k5-16
QVQLQESGGGLVQAGGSLRLSCAVSGNTLSRYAMGWFRQTPGKEREFVAAIRWNNAATYYADAVEGRFTISRDSGKNTVYLQMNNLKPEDTAVYYCAGRFLGYASSNAYHEALYNYDYWGQGTQVTVSS

SEQ ID NO: 146 - protein, 129 aa, Artificial
  CH1-7k5-17
QVQLQESGGGLVQAGGSLRLSCAVSGNTLSRYAMGWFRQTPGKEREFVAAIRWNNAATYYADSVEGRFTISRDNAKNTVYLQMNNLKPEDTAVYYCAGRFLGYASSNAYHEALYNYDYWGQGTQVTVSS

SEQ ID NO: 147 - protein, 129 aa, Artificial
  CH1-7k5-18
QVQLQESGGGLVQAGGSLRLSCAVSGNTLSRYAMGWFRQTPGKEREFVAAIRWNNAATYYADAVEGRFTISRDNAKNTVYLQMNNLKPEDTAVYYCAGRFLGYASSNAYHEALYNYDYWGQGTQVTVSS

SEQ ID NO: 148 - protein, 129 aa, Artificial
  CH1-7k5-19
QVQLQESGGGLVQAGGSLRLSCAVSGNTLSRYAMGWFRQTPGKEREFVAAIRWNNAATYYADAVEGRFTISRDTGKNTVYLQMNNLKPEDTAVYYCAGRFLGYASSNAYHEALYNYDYWGQGTQVTVSS

SEQ ID NO: 149 - protein, 129 aa, Artificial
  CH1-7k5-20
QVQLQESGGGLVQAGGSLRLSCAVSGNTLSRYAMGWFRQTPGKEREFVAAIRWNNAATYYAESVEGRFTISRDNAKNTVYLQMNNLKPEDTAVYYCAGRFLGYASSNAYHEALYNYDYWGQGTQVTVSS

SEQ ID NO: 150 - protein, 129 aa, Artificial
  CH1-7k5-21
QVQLQESGGGLVQAGGSLRLSCAVSGNTLSRYAMGWFRQTPGKEREFVAAIRWNEGATYYADSVEGRFTISRDSGKNTVYLQMNNLKPEDTAVYYCAGRFLGYASSNAYHEALYNYDYWGQGTQVTVSS

SEQ ID NO: 151 - protein, 129 aa, Artificial
  CH1-7k5-22
QVQLQESGGGLVQAGGSLRLSCAVSGNTLSRYAMGWFRQTPGKEREFVAAIRWNEGATYYAESVEGRFTISRDSGKNTVYLQMNNLKPEDTAVYYCAGRFLGYASSNAYHEALYNYDYWGQGTQVTVSS

SEQ ID NO: 152 - protein, 129 aa, Artificial
  CH1-7k5-23
QVQLQESGGGLVQAGGSLRLSCAVSGNTLSRYAMGWFRQTPGKEREFVAAIRWNEGATYYADSVEGRFTISRDTGKNTVYLQMNNLKPEDTAVYYCAGRFLGYASSNAYHEALYNYDYWGQGTQVTVSS

SEQ ID NO: 153 - protein, 129 aa, Artificial
  CH1-7k5-24
QVQLQESGGGLVQAGGSLRLSCAVSGNTLSRYAMGWFRQTPGKEREFVAAIRWNEGATYYAESVEGRFTISRDTGKNTVYLQMNNLKPEDTAVYYCAGRFLGYASSNAYHEALYNYDYWGQGTQVTVSS

SEQ ID NO: 154 - protein, 129 aa, Artificial
  CH1-7k5-25
QVQLQESGGGLVQAGGSLRLSCAVSGNTLSRYAMGWFRQTPGKEREFVAAIRWNEGATYYADAVEGRFTISRDSGKNTVYLQMNNLKPEDTAVYYCAGRFLGYASSNAYHEALYNYDYWGQGTQVTVSS

SEQ ID NO: 155 - protein, 129 aa, Artificial
  CH1-7k5-26
QVQLQESGGGLVQAGGSLRLSCAVSGNTLSRYAMGWFRQTPGKEREFVAAIRWNEGATYYADSVEGRFTISRDNAKNTVYLQMNNLKPEDTAVYYCAGRFLGYASSNAYHEALYNYDYWGQGTQVTVSS

SEQ ID NO: 156 - protein, 129 aa, Artificial
  CH1-7k5-27
QVQLQESGGGLVQAGGSLRLSCAVSGNTLSRYAMGWFRQTPGKEREFVAAIRWNEGATYYADAVEGRFTISRDNAKNTVYLQMNNLKPEDTAVYYCAGRFLGYASSNAYHEALYNYDYWGQGTQVTVSS

SEQ ID NO: 157 - protein, 129 aa, Artificial
  CH1-7k5-28
QVQLQESGGGLVQAGGSLRLSCAVSGNTLSRYAMGWFRQTPGKEREFVAAIRWNEGATYYADAVEGRFTISRDTGKNTVYLQMNNLKPEDTAVYYCAGRFLGYASSNAYHEALYNYDYWGQGTQVTVSS

SEQ ID NO: 158 - protein, 129 aa, Artificial
  CH1-7k5-29
QVQLQESGGGLVQAGGSLRLSCAVSGNTLSRYAMGWFRQTPGKEREFVAAIRWNEGATYYAESVEGRFTISRDNAKNTVYLQMNNLKPEDTAVYYCAGRFLGYASSNAYHEALYNYDYWGQGTQVTVSS

SEQ ID NO: 159 - protein, 9 aa, Artificial
  CDR-I
NTLSRYAMG

SEQ ID NO: 160 - protein, 9 aa, Artificial
  CDR-I
NTLSQYAMG

SEQ ID NO: 161 - protein, 9 aa, Artificial
  CDR-I
NTLSRYATG

SEQ ID NO: 162 - protein, 9 aa, Artificial
  CDR-I
NTLSPYAMG

SEQ ID NO: 163 - protein, 16 aa, Artificial
  CDR-II
AIRWNNGATYYADSVE

SEQ ID NO: 164 - protein, 16 aa, Artificial
  CDR-II
AIRWNNGATYYAESVE

SEQ ID NO: 165 - protein, 16 aa, Artificial
  CDR-II
AIRWNNGATYYADAVE

SEQ ID NO: 166 - protein, 16 aa, Artificial
  CDR-II
AIRWNNGATYYADSVK

SEQ ID NO: 167 - protein, 16 aa, Artificial
  CDR-II
AIRWNNGATYYAESVK

SEQ ID NO: 168 - protein, 16 aa, Artificial
  CDR-II
AIRWNNGATYYADAVK

SEQ ID NO: 169 - protein, 16 aa, Artificial
  CDR-II
AIRWNNGNTYYADSVK

SEQ ID NO: 170 - protein, 16 aa, Artificial
  CDR-II
AIRWNNGNTYYADSVE

SEQ ID NO: 171 - protein, 16 aa, Artificial
  CDR-II
AIRWNNGATYYADSVE

SEQ ID NO: 172 - protein, 16 aa, Artificial
  CDR-II
AIRWTNGNTYYADSVE

SEQ ID NO: 173 - protein, 16 aa, Artificial
  CDR-II
AIRWNSGHTYYADSVE

SEQ ID NO: 174 - protein, 16 aa, Artificial
  CDR-II
AIRWENGNTYYADSVE

SEQ ID NO: 175 - protein, 16 aa, Artificial
  CDR-II
PIRWNNGNTYYADSVE

SEQ ID NO: 176 - protein, 16 aa, Artificial
  CDR-II 176
AIRWNNAATYYADSVE

SEQ ID NO: 177 - protein, 16 aa, Artificial
  CDR-II 177
AIRWNNAATYYAESVE

SEQ ID NO: 178 - protein, 16 aa, Artificial
  CDR-II 178
AIRWNNAATYYADAVE

SEQ ID NO: 179 - protein, 16 aa, Artificial
  CDR-II 179
AIRWNEGATYYADSVE

SEQ ID NO: 180 - protein, 16 aa, Artificial
  CDR-II 180
AIRWNEGATYYAESVE

SEQ ID NO: 181 - protein, 16 aa, Artificial
  CDR-II 181
AIRWNEGATYYADAVE

SEQ ID NO: 182 - protein, 20 aa, Artificial
  CDR-III
RFLGYASSNAYHEALYNYDY

SEQ ID NO: 183 - protein, 20 aa, Artificial
  CDR-III
RFLPYASSNAYHEALYNYDY

SEQ ID NO: 184 - protein, 20 aa, Artificial
  CDR-III
RFLPYASSNAYHESLYNYDY

SEQ ID NO: 185 - protein, 20 aa, Artificial
  CDR-III
RFLPYASSNAYHETLYNYDY

SEQ ID NO: 186 - protein, 26 aa, Artificial
  FR1
QVQLQESGGGLVQAGGSLRLSCAVSG

SEQ ID NO: 187 - protein, 14 aa, Artificial
  FR2
WFRQTPGNEREFVA

SEQ ID NO: 188 - protein, 33 aa, Artificial
  FR3
GRFTISRDSGKNTVYLQMNNLKPEDTAVYYCAG

SEQ ID NO: 189 - protein, 11 aa, Artificial
  FR4
WGQGTQVTVSS

SEQ ID NO: 190 - protein, 98 aa, Artificial
  Human IgG1 CH1
ASTKGPSVFPLAPSSKSTSGGTAALGCLVKDYFPEPVTVSWNSGALTSGVHTFPAVLQSSGLYSLSSVVTVPSSSLGTQTYICNVNHKPSNTKVDKKV

SEQ ID NO: 191 - protein, 98 aa, Artificial
  Human IgG2 CH1
ASTKGPSVFPLAPCSRSTSESTAALGCLVKDYFPEPVTVSWNSGALTSGVHTFPAVLQSSGLYSLSSVVTVPSSNFGTQTYTCNVDHKPSNTKVDKTV

SEQ ID NO: 192 - protein, 98 aa, Artificial
  Human IgG3 CH1
ASTKGPSVFPLAPCSRSTSGGTAALGCLVKDYFPEPVTVSWNSGALTSGVHTFPAVLQSSGLYSLSSVVTVPSSSLGTQTYTCNVNHKPSNTKVDKRV

SEQ ID NO: 193 - protein, 98 aa, Artificial
  Human IgG4 CH1
ASTKGPSVFPLAPCSRSTSESTAALGCLVKDYFPEPVTVSWNSGALTSGVHTFPAVLQSSGLYSLSSVVTVPSSSLGTKTYTCNVDHKPSNTKVDKRV

SEQ ID NO: 194 - protein, 97 aa, Artificial
  Baboon IgG1 CH1
ASTKGPSVFPLAPSSRSTSESTAALGCLVKDYFPEPVTVSWNSGSLTSGVHTFPAVLQSSGLYSLSSVVTVPSSSLGQTYVCNVNHKPSNTKVDKKV

SEQ ID NO: 195 - protein, 98 aa, Artificial
  Chimpanzee IgG CH1
ASTKGPSVFPLAPSSKSTSGGTQALGCLVKDYFPEPVTVSWNSGALTSGVHTFPAVLQSSGLYSLSSVVTVPSSSLGTQTYICNVDHKPSNTKVDKKV

SEQ ID NO: 196 - protein, 98 aa, Artificial
  Rhesus IgG CH1
ASTKGPSVFPLAPSSRSTSESTAALGCLVKDYFPEPVTVSWNSGSLTSGVHTFPAVLQSSGLYSLSSVVTVPSSSLGTQTYVCNVNHKPSNTKVDKRV

SEQ ID NO: 197 - protein, 98 aa, Artificial
  Cat IgG1 CH1
ASTTAPSVFPLAPSCGTTSGATVALACLVLGYFPEPVTVSWNSGALTSGVHTFPAVLQASGLYSLSSMVTVPSSRWLSDTFTCNVAHPPSNTKVDKTV

SEQ ID NO: 198 - protein, 98 aa, Artificial
  Dog IgG (A) CH1
ASTTAPSVFPLAPSCGSTSGSTVALACLVSGYFPEPVTVSWNSGSLTSGVHTFPSVLQSSGLHSLSSMVTVPSSRWPSETFTCNVVHPASNTKVDKPV

SEQ ID NO: 199 - protein, 94 aa, Artificial
  Guinea Pig IgG2 CH1
ARTTAPSVFPLAASCVDTSGSMMTLGCLVKGYFPEPVTVKWNSGALTSGVHTFPAVLQSGLYSLTSMVTVPSSQKKATCNVAHPASSTKVDKTV

SEQ ID NO: 200 - protein, 98 aa, Artificial
  Horse IgG1 CH1
ASTTAPKVFALAPGCGTTSDSTVALGCLVSGYFPEPVKVSWNSGSLTSGVHTFPSVLQSSGFYSLSSMVTVPASTWTSETYICNVVHAASNFKVDKRI

SEQ ID NO: 201 - protein, 95 aa, Artificial
  Rabbit IgG CH1
GQPKAPSVFPLAPCCGDTPSSTVTLGCLVKGYLPEPVTVTWNSGTLTNGVRTFPSVRQSSGLYSLSSVVSVTSSSQPVTCNVAHPATNTKVDKTV

SEQ ID NO: 202 - protein, 98 aa, Artificial
  Swine IgG1 CH1
APKTAPSVYPLAPCGRDTSGPNVALGCLASSYFPEPVTVTWNSGALTSGVHTFPSVLQPSGLYSLSSMVTVPASSLSSKSYTCNVNHPATTTKVDKRV

SEQ ID NO: 203 - protein, 98 aa, Artificial
  Swine IgG2 CH1
APKTAPSVYPLAPCGRDVSGPNVALGCLASSYFPEPVTVTWNSGALTSGVHTFPSVLQPSGLYSLSSMVTVPASSLSSKSYTCNVNHPATTTKVDKRV

SEQ ID NO: 204 - protein, 96 aa, Artificial
  Bovine IgG1 CH1
ASTTAPKVYPLSSCCGDKSSSTVTLGCLVSSYMPEPVTVTWNSGALKSGVHTFPAVLQSSGLYSLSSMVTVPASSSGTQTFTCNVAHPASSTKVDK

SEQ ID NO: 205 - protein, 96 aa, Artificial
  Bovine IgG2 CH1
ASTTAPKVYPLSSCCGDKSSSGVTLGCLVSSYMPEPVTVTWNSGALKSGVHTFPAVLQSSGLYSLSSMVTVPASSSGTQTFTCNVAHPASSTKVDK

SEQ ID NO: 206 - protein, 98 aa, Artificial
  Sheep IgG1 CH1
ASTTPPKVYPLTSCCGDTSSSIVTLGCLVSSYMPEPVTVTWNSGALTSGVHTFPAILQSSGLYSLSSVVTVPASTSGAQTFICNVAHPASSTKVDKRV

SEQ ID NO: 207 - protein, 98 aa, Artificial
  Goat IgG1 CH1
ASTTPPKVYPLTSCCGDTSSSIVTLGCLVSSYMPEPVTVTWNSGALTSGVHTFPAVLQSSGLYSLSSMVTVPASTSGAQTFICNVAHPASSTKVDKRV

SEQ ID NO: 208 - protein, 98 aa, Artificial
  Llama IgG1a CH1
ASTKAPSVYPLTARCGDTPGSTVAFGCLVWGYIPEPVTVTWNSGALSSGVHTFPSVFMSSGLYTLSSLVTMPASSSTGKTFICNVAHPASSTKVDKRV

SEQ ID NO: 209 - protein, 98 aa, Artificial
  Llama IgG1b CH1
ASTKAPSVYPLTARCGDTPGSTVAFGCLVWGYIPEPVTVTWNSGALSSGVHTFPSVFMSSGLYSLSSLVTLPTSSSTGKTFICNVAHPASSTKVDKRV

SEQ ID NO: 210 - protein, 97 aa, Artificial
  Rat IgG1 CH1
AETTAPSVYPLAPGTALKSNSMVTLGCLVKGYFPEPVTVTWNSGALSSGVHTFPAVLQSGLYTLTSSVTVPSSTWPSQTVTCNVAHPASSTKVDKKI

SEQ ID NO: 211 - protein, 97 aa, Artificial
  Rat IgG2a CH1
AETTAPSVYPLAPGTALKSNSMVTLGCLVKGYFPEPVTVTWNSGALSSGVHTFPAVLQSGLYTLTSSVTVPSSTWSSQAVTCNVAHPASSTKVDKKI

SEQ ID NO: 212 - protein, 95 aa, Artificial
  Rat IgG2b CH1
AQTTAPSVYPLAPGCGDTTSSTVTLGCLVKGYFPEPVTVTWNSGALSSDVHTFPAVLQSGLYTLTSSVTSSTWPSQTVTCNVAHPASSTKVDKKV

SEQ ID NO: 213 - protein, 97 aa, Artificial
  Rat IgG2c CH1
ARTTAPSVYPLVPGCSGTSGSLVTLGCLVKGYFPEPVTVKWNSGALSSGVHTFPAVLQSGLYTLSSSVTVPSSTWSSQTVTCSVAHPATKSNLIKRI

SEQ ID NO: 214 - protein, 97 aa, Artificial
  Mouse IgG1 CH1
AKTTPPSVYPLAPGSAAQTNSMVTLGCLVKGYFPEPVTVTWNSGSLSSGVHTFPAVLQSDLYTLSSSVTVPSSPRPSETVTCNVAHPASSTKVDKKI

SEQ ID NO: 215 - protein, 97 aa, Artificial
  Mouse IgG2a CH1
AKTTAPSVYPLAPVCGDTTGSSVTLGCLVKGYFPEPVTLTWNSGSLSSGVHTFPAVLQSDLYTLSSSVTVTSSTWPSQSITCNVAHPASSTKVDKKI

SEQ ID NO: 216 - protein, 97 aa, Artificial
  Mouse IgG2b CH1
AKTTPPSVYPLAPGCGDTTGSSVTLGCLVKGYFPESVTVTWNSGSLSSSVHTFPALLQSGLYTMSSSVTVPSSTWPSQTVTCSVAHPASSTTVDKKL

SEQ ID NO: 217 - protein, 97 aa, Artificial
  Mouse IgG3 CH1
ATTTAPSVYPLVPGCSDTSGSSVTLGCLVKGYFPEPVTVKWNYGALSSGVRTVSSVLQSGFYSLSSLVTVPSSTWPSQTVICNVAHPASKTELIKRI